European Patent Application EP 4 361 267 A1, published May 1, 2024. Title: Method for identifying T cell epitope sequences and its application. Applicant: Repertoire Genesis Incorporation. The sequence listing filed with the application follows.

SEQUENCE LISTING (501 sequences)

SEQ ID NO: 1 - protein, 15 aa, Homo sapiens
ITMDWTWRFLFVVAA

SEQ ID NO: 2 - protein, 15 aa, Homo sapiens
TMDWTWRFLFVVAAA

SEQ ID NO: 3 - protein, 15 aa, Homo sapiens
MDWTWRFLFVVAAAT

SEQ ID NO: 4 - protein, 15 aa, Homo sapiens
DWTWRFLFVVAAATG

SEQ ID NO: 5 - protein, 15 aa, Homo sapiens
WTWRFLFVVAAATGV

SEQ ID NO: 6 - protein, 15 aa, Homo sapiens
TWRFLFVVAAATGVQ

SEQ ID NO: 7 - protein, 15 aa, Homo sapiens
WRFLFVVAAATGVQS

SEQ ID NO: 8 - protein, 15 aa, Homo sapiens
RFLFVVAAATGVQSQ

SEQ ID NO: 9 - protein, 15 aa, Homo sapiens
FLFVVAAATGVQSQV

SEQ ID NO: 10 - protein, 15 aa, Homo sapiens
LFVVAAATGVQSQVQ

SEQ ID NO: 11 - protein, 15 aa, Homo sapiens
FVVAAATGVQSQVQL

SEQ ID NO: 12 - protein, 15 aa, Homo sapiens
VVAAATGVQSQVQLV

SEQ ID NO: 13 - protein, 15 aa, Homo sapiens
VAAATGVQSQVQLVQ

SEQ ID NO: 14 - protein, 15 aa, Homo sapiens
AAATGVQSQVQLVQS

SEQ ID NO: 15 - protein, 15 aa, Homo sapiens
AATGVQSQVQLVQSG

SEQ ID NO: 16 - protein, 15 aa, Homo sapiens
ATGVQSQVQLVQSGA

SEQ ID NO: 17 - protein, 15 aa, Homo sapiens
TGVQSQVQLVQSGAE

SEQ ID NO: 18 - protein, 15 aa, Homo sapiens
GVQSQVQLVQSGAEV

SEQ ID NO: 19 - protein, 15 aa, Homo sapiens
VQSQVQLVQSGAEVK

SEQ ID NO: 20 - protein, 15 aa, Homo sapiens
QSQVQLVQSGAEVKK

SEQ ID NO: 21 - protein, 15 aa, Homo sapiens
SQVQLVQSGAEVKKP

SEQ ID NO: 22 - protein, 15 aa, Homo sapiens
QVQLVQSGAEVKKPG

SEQ ID NO: 23 - protein, 15 aa, Homo sapiens
VQLVQSGAEVKKPGS

SEQ ID NO: 24 - protein, 15 aa, Homo sapiens
QLVQSGAEVKKPGSS

SEQ ID NO: 25 - protein, 15 aa, Homo sapiens
LVQSGAEVKKPGSSV

SEQ ID NO: 26 - protein, 15 aa, Homo sapiens
VQSGAEVKKPGSSVK

SEQ ID NO: 27 - protein, 15 aa, Homo sapiens
QSGAEVKKPGSSVKV

SEQ ID NO: 28 - protein, 15 aa, Homo sapiens
SGAEVKKPGSSVKVS

SEQ ID NO: 29 - protein, 15 aa, Homo sapiens
GAEVKKPGSSVKVSC

SEQ ID NO: 30 - protein, 15 aa, Homo sapiens
AEVKKPGSSVKVSCK

SEQ ID NO: 31 - protein, 15 aa, Homo sapiens
EVKKPGSSVKVSCKA

SEQ ID NO: 32 - protein, 15 aa, Homo sapiens
VKKPGSSVKVSCKAT

SEQ ID NO: 33 - protein, 15 aa, Homo sapiens
KKPGSSVKVSCKATG

SEQ ID NO: 34 - protein, 15 aa, Homo sapiens
KPGSSVKVSCKATGG

SEQ ID NO: 35 - protein, 15 aa, Homo sapiens
PGSSVKVSCKATGGT

SEQ ID NO: 36 - protein, 15 aa, Homo sapiens
GSSVKVSCKATGGTF

SEQ ID NO: 37 - protein, 15 aa, Homo sapiens
SSVKVSCKATGGTFS

SEQ ID NO: 38 - protein, 15 aa, Homo sapiens
SVKVSCKATGGTFSS

SEQ ID NO: 39 - protein, 15 aa, Homo sapiens
VKVSCKATGGTFSSY

SEQ ID NO: 40 - protein, 15 aa, Homo sapiens
KVSCKATGGTFSSYA

SEQ ID NO: 41 - protein, 15 aa, Homo sapiens
VSCKATGGTFSSYAI

SEQ ID NO: 42 - protein, 15 aa, Homo sapiens
SCKATGGTFSSYAIS

SEQ ID NO: 43 - protein, 15 aa, Homo sapiens
CKATGGTFSSYAISW

SEQ ID NO: 44 - protein, 15 aa, Homo sapiens
KATGGTFSSYAISWV

SEQ ID NO: 45 - protein, 15 aa, Homo sapiens
ATGGTFSSYAISWVR

SEQ ID NO: 46 - protein, 15 aa, Homo sapiens
TGGTFSSYAISWVRQ

SEQ ID NO: 47 - protein, 15 aa, Homo sapiens
GGTFSSYAISWVRQT

SEQ ID NO: 48 - protein, 15 aa, Homo sapiens
GTFSSYAISWVRQTP

SEQ ID NO: 49 - protein, 15 aa, Homo sapiens
TFSSYAISWVRQTPG

SEQ ID NO: 50 - protein, 15 aa, Homo sapiens
FSSYAISWVRQTPGQ

SEQ ID NO: 51 - protein, 15 aa, Homo sapiens
SSYAISWVRQTPGQG

SEQ ID NO: 52 - protein, 15 aa, Homo sapiens
SYAISWVRQTPGQGL

SEQ ID NO: 53 - protein, 15 aa, Homo sapiens
YAISWVRQTPGQGLE

SEQ ID NO: 54 - protein, 15 aa, Homo sapiens
AISWVRQTPGQGLEW

SEQ ID NO: 55 - protein, 15 aa, Homo sapiens
ISWVRQTPGQGLEWM

SEQ ID NO: 56 - protein, 15 aa, Homo sapiens
SWVRQTPGQGLEWMG

SEQ ID NO: 57 - protein, 15 aa, Homo sapiens
WVRQTPGQGLEWMGG

SEQ ID NO: 58 - protein, 15 aa, Homo sapiens
VRQTPGQGLEWMGGR

SEQ ID NO: 59 - protein, 15 aa, Homo sapiens
RQTPGQGLEWMGGRI

SEQ ID NO: 60 - protein, 15 aa, Homo sapiens
QTPGQGLEWMGGRIP

SEQ ID NO: 61 - protein, 15 aa, Homo sapiens
TPGQGLEWMGGRIPI

SEQ ID NO: 62 - protein, 15 aa, Homo sapiens
PGQGLEWMGGRIPIF

SEQ ID NO: 63 - protein, 15 aa, Homo sapiens
GQGLEWMGGRIPIFG

SEQ ID NO: 64 - protein, 15 aa, Homo sapiens
QGLEWMGGRIPIFGI

SEQ ID NO: 65 - protein, 15 aa, Homo sapiens
GLEWMGGRIPIFGIP

SEQ ID NO: 66 - protein, 15 aa, Homo sapiens
LEWMGGRIPIFGIPD

SEQ ID NO: 67 - protein, 15 aa, Homo sapiens
EWMGGRIPIFGIPDY

SEQ ID NO: 68 - protein, 15 aa, Homo sapiens
WMGGRIPIFGIPDYA

SEQ ID NO: 69 - protein, 15 aa, Homo sapiens
MGGRIPIFGIPDYAQ

SEQ ID NO: 70 - protein, 15 aa, Homo sapiens
GGRIPIFGIPDYAQK

SEQ ID NO: 71 - protein, 15 aa, Homo sapiens
GRIPIFGIPDYAQKF

SEQ ID NO: 72 - protein, 15 aa, Homo sapiens
RIPIFGIPDYAQKFQ

SEQ ID NO: 73 - protein, 15 aa, Homo sapiens
IPIFGIPDYAQKFQG

SEQ ID NO: 74 - protein, 15 aa, Homo sapiens
PIFGIPDYAQKFQGR

SEQ ID NO: 75 - protein, 15 aa, Homo sapiens
IFGIPDYAQKFQGRV

SEQ ID NO: 76 - protein, 15 aa, Homo sapiens
FGIPDYAQKFQGRVT

SEQ ID NO: 77 - protein, 15 aa, Homo sapiens
GIPDYAQKFQGRVTI

SEQ ID NO: 78 - protein, 15 aa, Homo sapiens
IPDYAQKFQGRVTIT

SEQ ID NO: 79 - protein, 15 aa, Homo sapiens
PDYAQKFQGRVTITA

SEQ ID NO: 80 - protein, 15 aa, Homo sapiens
DYAQKFQGRVTITAD

SEQ ID NO: 81 - protein, 15 aa, Homo sapiens
YAQKFQGRVTITADE

SEQ ID NO: 82 - protein, 15 aa, Homo sapiens
AQKFQGRVTITADES

SEQ ID NO: 83 - protein, 15 aa, Homo sapiens
QKFQGRVTITADEST

SEQ ID NO: 84 - protein, 15 aa, Homo sapiens
KFQGRVTITADESTT

SEQ ID NO: 85 - protein, 15 aa, Homo sapiens
FQGRVTITADESTTT

SEQ ID NO: 86 - protein, 15 aa, Homo sapiens
QGRVTITADESTTTG

SEQ ID NO: 87 - protein, 9 aa, Homo sapiens
ITMDWTWRF

SEQ ID NO: 88 - protein, 9 aa, Homo sapiens
TMDWTWRFL

SEQ ID NO: 89 - protein, 9 aa, Homo sapiens
MDWTWRFLF

SEQ ID NO: 90 - protein, 9 aa, Homo sapiens
DWTWRFLFV

SEQ ID NO: 91 - protein, 9 aa, Homo sapiens
WTWRFLFVV

SEQ ID NO: 92 - protein, 9 aa, Homo sapiens
TWRFLFVVA

SEQ ID NO: 93 - protein, 9 aa, Homo sapiens
WRFLFVVAA

SEQ ID NO: 94 - protein, 9 aa, Homo sapiens
RFLFVVAAA

SEQ ID NO: 95 - protein, 9 aa, Homo sapiens
FLFVVAAAT

SEQ ID NO: 96 - protein, 9 aa, Homo sapiens
LFVVAAATG

SEQ ID NO: 97 - protein, 9 aa, Homo sapiens
FVVAAATGV

SEQ ID NO: 98 - protein, 9 aa, Homo sapiens
VVAAATGVQ

SEQ ID NO: 99 - protein, 9 aa, Homo sapiens
VAAATGVQS

SEQ ID NO: 100 - protein, 9 aa, Homo sapiens
AAATGVQSQ

SEQ ID NO: 101 - protein, 9 aa, Homo sapiens
AATGVQSQV

SEQ ID NO: 102 - protein, 9 aa, Homo sapiens
ATGVQSQVQ

SEQ ID NO: 103 - protein, 9 aa, Homo sapiens
TGVQSQVQL

SEQ ID NO: 104 - protein, 9 aa, Homo sapiens
GVQSQVQLV

SEQ ID NO: 105 - protein, 9 aa, Homo sapiens
VQSQVQLVQ

SEQ ID NO: 106 - protein, 9 aa, Homo sapiens
QSQVQLVQS

SEQ ID NO: 107 - protein, 9 aa, Homo sapiens
SQVQLVQSG

SEQ ID NO: 108 - protein, 9 aa, Homo sapiens
QVQLVQSGA

SEQ ID NO: 109 - protein, 9 aa, Homo sapiens
VQLVQSGAE

SEQ ID NO: 110 - protein, 9 aa, Homo sapiens
QLVQSGAEV

SEQ ID NO: 111 - protein, 9 aa, Homo sapiens
LVQSGAEVK

SEQ ID NO: 112 - protein, 9 aa, Homo sapiens
VQSGAEVKK

SEQ ID NO: 113 - protein, 9 aa, Homo sapiens
QSGAEVKKP

SEQ ID NO: 114 - protein, 9 aa, Homo sapiens
SGAEVKKPG

SEQ ID NO: 115 - protein, 9 aa, Homo sapiens
GAEVKKPGS

SEQ ID NO: 116 - protein, 9 aa, Homo sapiens
AEVKKPGSS

SEQ ID NO: 117 - protein, 9 aa, Homo sapiens
EVKKPGSSV

SEQ ID NO: 118 - protein, 9 aa, Homo sapiens
VKKPGSSVK

SEQ ID NO: 119 - protein, 9 aa, Homo sapiens
KKPGSSVKV

SEQ ID NO: 120 - protein, 9 aa, Homo sapiens
KPGSSVKVS

SEQ ID NO: 121 - protein, 9 aa, Homo sapiens
PGSSVKVSC

SEQ ID NO: 122 - protein, 9 aa, Homo sapiens
GSSVKVSCK

SEQ ID NO: 123 - protein, 9 aa, Homo sapiens
SSVKVSCKA

SEQ ID NO: 124 - protein, 9 aa, Homo sapiens
SVKVSCKAT

SEQ ID NO: 125 - protein, 9 aa, Homo sapiens
VKVSCKATG

SEQ ID NO: 126 - protein, 9 aa, Homo sapiens
KVSCKATGG

SEQ ID NO: 127 - protein, 9 aa, Homo sapiens
VSCKATGGT

SEQ ID NO: 128 - protein, 9 aa, Homo sapiens
SCKATGGTF

SEQ ID NO: 129 - protein, 9 aa, Homo sapiens
CKATGGTFS

SEQ ID NO: 130 - protein, 9 aa, Homo sapiens
KATGGTFSS

SEQ ID NO: 131 - protein, 9 aa, Homo sapiens
ATGGTFSSY

SEQ ID NO: 132 - protein, 9 aa, Homo sapiens
TGGTFSSYA

SEQ ID NO: 133 - protein, 9 aa, Homo sapiens
GGTFSSYAI

SEQ ID NO: 134 - protein, 9 aa, Homo sapiens
GTFSSYAIS

SEQ ID NO: 135 - protein, 9 aa, Homo sapiens
TFSSYAISW

SEQ ID NO: 136 - protein, 9 aa, Homo sapiens
FSSYAISWV

SEQ ID NO: 137 - protein, 9 aa, Homo sapiens
SSYAISWVR

SEQ ID NO: 138 - protein, 9 aa, Homo sapiens
SYAISWVRQ

SEQ ID NO: 139 - protein, 9 aa, Homo sapiens
YAISWVRQT

SEQ ID NO: 140 - protein, 9 aa, Homo sapiens
AISWVRQTP

SEQ ID NO: 141 - protein, 9 aa, Homo sapiens
ISWVRQTPG

SEQ ID NO: 142 - protein, 9 aa, Homo sapiens
SWVRQTPGQ

SEQ ID NO: 143 - protein, 9 aa, Homo sapiens
WVRQTPGQG

SEQ ID NO: 144 - protein, 9 aa, Homo sapiens
VRQTPGQGL

SEQ ID NO: 145 - protein, 9 aa, Homo sapiens
RQTPGQGLE

SEQ ID NO: 146 - protein, 9 aa, Homo sapiens
QTPGQGLEW

SEQ ID NO: 147 - protein, 9 aa, Homo sapiens
TPGQGLEWM

SEQ ID NO: 148 - protein, 9 aa, Homo sapiens
PGQGLEWMG

SEQ ID NO: 149 - protein, 9 aa, Homo sapiens
GQGLEWMGG

SEQ ID NO: 150 - protein, 9 aa, Homo sapiens
QGLEWMGGR

SEQ ID NO: 151 - protein, 9 aa, Homo sapiens
GLEWMGGRI

SEQ ID NO: 152 - protein, 9 aa, Homo sapiens
LEWMGGRIP

SEQ ID NO: 153 - protein, 9 aa, Homo sapiens
EWMGGRIPI

SEQ ID NO: 154 - protein, 9 aa, Homo sapiens
WMGGRIPIF

SEQ ID NO: 155 - protein, 9 aa, Homo sapiens
MGGRIPIFG

SEQ ID NO: 156 - protein, 9 aa, Homo sapiens
GGRIPIFGI

SEQ ID NO: 157 - protein, 9 aa, Homo sapiens
GRIPIFGIP

SEQ ID NO: 158 - protein, 9 aa, Homo sapiens
RIPIFGIPD

SEQ ID NO: 159 - protein, 9 aa, Homo sapiens
IPIFGIPDY

SEQ ID NO: 160 - protein, 9 aa, Homo sapiens
PIFGIPDYA

SEQ ID NO: 161 - protein, 9 aa, Homo sapiens
IFGIPDYAQ

SEQ ID NO: 162 - protein, 9 aa, Homo sapiens
FGIPDYAQK

SEQ ID NO: 163 - protein, 9 aa, Homo sapiens
GIPDYAQKF

SEQ ID NO: 164 - protein, 9 aa, Homo sapiens
IPDYAQKFQ

SEQ ID NO: 165 - protein, 9 aa, Homo sapiens
PDYAQKFQG

SEQ ID NO: 166 - protein, 9 aa, Homo sapiens
DYAQKFQGR

SEQ ID NO: 167 - protein, 9 aa, Homo sapiens
YAQKFQGRV

SEQ ID NO: 168 - protein, 9 aa, Homo sapiens
AQKFQGRVT

SEQ ID NO: 169 - protein, 9 aa, Homo sapiens
QKFQGRVTI

SEQ ID NO: 170 - protein, 9 aa, Homo sapiens
KFQGRVTIT

SEQ ID NO: 171 - protein, 9 aa, Homo sapiens
FQGRVTITA

SEQ ID NO: 172 - protein, 9 aa, Homo sapiens
QGRVTITAD

SEQ ID NO: 173 - protein, 181 aa, Homo sapiens
MDWTWSILLLVAAATGAHSQGQLVQSGPEVMKPGASVKVSCQASGYTFTTYGISWVRQAPGQGLEWMGLISPRNGNTNYAQTFQGRVTVTTDTSTNTAYMELRSLRSDDTAVYYCARTRRDPDGMDVWGQGTTVTVSSASTKGPSVFPLAPCSRSTSESTAALGCLVKDYFPEPVTVSWNS

SEQ ID NO: 174 - protein, 182 aa, Homo sapiens
MEFGLSWLFLVAILKGVQCEVQLLESGGGLVQPGGSLRLSCAASGFTFSSYSMTWVRQAPGKGLEWVSAISDSGRETYYADSVKGHFTISRDNSKNTVFLQMNSLRAEDTAVYYCAREMTRFYPLFEYWGQGTLVTVSSASTKGPSVFPLAPSSKSTSGGTAALGCLVKDYFPEPVTVSWNS

SEQ ID NO: 175 - protein, 123 aa, Homo sapiens
IPLEWISLISWDGSSTHYADSVKGRFTISRDNSKNSLYLQMSGLRTGDTAFYYCVKDSLAATGRSNFHSWGQGTLVTVSSASTKGPSVFPLAPCSRSTSESTAALGCLVKDYFPEPVTVSWNS

SEQ ID NO: 176 - protein, 114 aa, Homo sapiens
HPGDSDLRYSPSLQGQVTISVDSSISTAYLQWASLKASDTAIYYCARQGYYDDNGHFRDYWGQGTLITVSSASTKGPSVFPLAPCSRSTSESTAALGCLVKDYFPEPVTVSWNS

SEQ ID NO: 177 - protein, 188 aa, Homo sapiens
MDPLHKNMKHLWFFLLLVAAPRWVLSQVQLQESGPGAVKPSETLSLTCNVSGGSMTTYYWSWIRQSPEKGLEWIGFISDSGHANYSPSLKSRVTISVDTSKNQFSLRLTSVTAADTALYYCARATSRSRGWFDPWGQGTLVTITSPSTKGPSVFPLAPCSRSTSESTAALGCLVKDYFPEPVTVSWNS

SEQ ID NO: 178 - protein, 192 aa, Homo sapiens
MEFGLSWIFLAAILKGVQCEVQLVESGGGLVKPGGSLRLSCAASGFTFSNAWMTWVRQAPGKGLEWVGRIKSKTDGGTTDYAAPVKGRFTISRDDSKNTLYLQMNSLKTEDTAVYYCTTEIMITFGGVIATGGYGMDVWGQGTTVTVSSASTKGPSVFPLAPSSKSTSGGTAALGCLVKDYFPEPVTVSWNS

SEQ ID NO: 179 - protein, 101 aa, Homo sapiens
ETANTTPNSHSKNTLNLQMNSLRAEDTAVYFCAKDPFFRTRTEYFQDWGQGTLVIVSSASTKGPSVFPLAPSSKSTSGGTAALGCLVKDYFPEPVTVSWNS

SEQ ID NO: 180 - protein, 175 aa, Homo sapiens
MGSTAILALLLAVLQGACAEVQLMQSGAEVKKPGESLKISCKGSGYRFSIFWIGWVRQMPGKGLEWMGIIYPSDSDTRYNPSLQGQATFSVDKSINTAYLQWSSLKASDTAMYYCTRQYDIWGQGTMVTVSPPSTKGPSVFPLAPSSKSTSGGTAALGCLVKDYFPEPVTVSWNS

SEQ ID NO: 181 - protein, 185 aa, Homo sapiens
MDPLHKNMKHLWFFLLLVAAPRWVLSQVQLQESGPGLVKPSETLSLTCTVSGASISRYYWSWIRQPAGKGLEWIGRMYTSGTTDYNPSLKNRVTMSVDTSNNQFSLNLRSVTAADTAKYYCTRGGSYFLDYWGRGILVTVSSASTKGPSVFPLAPCSRSTSESTAALGCLVKDYFPEPVTVSWNS

SEQ ID NO: 182 - protein, 188 aa, Homo sapiens
MDWTWRILFLVAAVTSAHSQVQLVQSGAEVKRPGASVKVSCKAFGYSFTSNDMNWVRQAPGQGLEWMGSVSPSSGTTVYAPRFQDRVTMTRDTSIGTAYMELSSLRYDDTAVYYCARGVFSGSGLGQYYYAMDVWGQGTTVTVSSASTKGPSVFPLAPSSKSTSGGTAALGCLVKDYFPEPVTVSWNS

SEQ ID NO: 183 - protein, 188 aa, Homo sapiens
MDWTWRFLFVVAAATGVQSQVQLVQSGAEVKKPGSSVKVSCKATGGTFSSYAISWVRQTPGQGLEWMGGRIPIFGIPDYAQKFQGRVTITADESTTTGYMELSNLRSEDTAVYYCASGTYYYGSGSHGFGAFDIWGQGTMVTVSSASTKGPSVFPLAPSSKSTSGGTAALGCLVKDYFPEPVTVSWNS

SEQ ID NO: 184 - protein, 178 aa, Homo sapiens
MELGLSWVFLVAILEGVQCEVQLVESGGGLVQPGGSLGLSCAASGFIFTDYWMHWVRQAPGKGLEWVANIKQDGSVKYYLDSVKGRFTVSRDNTKKSLSLQMDSLRVDDTAVYYCVRDPYREGCWGQGTLVTVSSASTKGPSVFPLAPCSRSTSESTAALGCLVKDYFPEPVTVSWNS

SEQ ID NO: 185 - protein, 181 aa, Homo sapiens
MKHLWFFLLLVAAPRWVLSQVQLQQWGAGLLKPSETLSLTCAVNAGSFSGYYWSWIRQPPGKGLEWIGNIKHSGSTKSNPSLQSRVTISVDSSKKQFSLKLNSVTAADTALYYCARGWGKLGSILDIWGQGTMVTVSSASTKGPSVFPLAPSSKSTSGGTAALGCLVKDYFPEPVTVSWNS

SEQ ID NO: 186 - protein, 186 aa, Homo sapiens
MEFGLSWVFLVALLRGVQCQVQLVESGGGVVQPGRSLRLSCAASGFTFSAYGMHWVRQSPGKGLEWVALISYDGSEKYRDSVKGRFTISRDISKNTLYLQMNSLRPEDTAVYYCAKDLISNELYSSTWPPGFWGQGTLVTVSSASTKGPSVFPLAPSSKSTSGGTAALGCLVKDYFPEPVTVSWNS

SEQ ID NO: 187 - protein, 84 aa, Homo sapiens
VVLTMTNTDPVDTGTYWCSHSHGDTYGMGVWGQGTRVTVSSASTKGPSVFPLAPCSRSTSESTAALGCLVKDYFPEPVTVSWNS

SEQ ID NO: 188 - protein, 183 aa, Homo sapiens
MEFGLSWVFLVVILQGVQCEVQLVESGGGLVQPGGSLRLSCAASGFTLSDHFMDWVRQAPGKGLEWVGRTRDEADNFITDYAASVKGRFTISRDDLKNSVYLQMNTLTTEDTGVYYCTRGFQWGDGFDSWGQGTLVTVSSASTKGPSVFPLAPCSRSTSESTAALGCLVKDYFPEPVTVSWNS

SEQ ID NO: 189 - protein, 186 aa, Homo sapiens
MEFGLSWVFLVTILKGVQCEVQLAESGGGLVQPGGSLRLSCAVSGFTVSNNFMTWVRQAPGKGLEWVSVVYPGGMTYYADSVKGRFTISRDNFENALYLQMNSLRSEDTAIYYCARGDSWSGYSFPFHAFDIWGQGTMVTVSSASTKGPSVFPLAPSSKSTSGGTAALGCLVKDYFPEPVTVSWNS

SEQ ID NO: 190 - protein, 183 aa, Homo sapiens
MELGLRWVFLVAILEGVQCEVLLVESGGGLVKPGGSLRLSCAASGFSFSRYSMSWVRQAPGKGLEWVSSITSSSAYIYYADSVKGRFTVSRDNTEISLYLQMNSLRAEDTAVYYCVTPLNSGMTTAFHIWGQGTLVTVSSASTKGPSVFPLAPSSKSTSGGTAALGCLVKDYFPEPVTVSWNS

SEQ ID NO: 191 - protein, 84 aa, Homo sapiens
SVTAADTANYFCAREVLWFRAFPHSDAFDIWGQGTMVTVSSASTKGPSVFPLAPSSKSTSGGTAALGCLVKDYFPEPVTVSWNS

SEQ ID NO: 192 - protein, 84 aa, Homo sapiens
DTATYYCARIHRAYYDILTGYYFYYYGMDVWGQGTTVTVSSASTKGPSVFPLAPCSRSTSESTAALGCLVKDYFPEPVTVSWNS

SEQ ID NO: 193 - protein, 9 aa, Homo sapiens
SGHIPPLKK

SEQ ID NO: 194 - protein, 9 aa, Homo sapiens
GHIPPLKKP

SEQ ID NO: 195 - protein, 9 aa, Homo sapiens
HIPPLKKPL

SEQ ID NO: 196 - protein, 9 aa, Homo sapiens
IPPLKKPLG

SEQ ID NO: 197 - protein, 9 aa, Homo sapiens
PPLKKPLGA

SEQ ID NO: 198 - protein, 9 aa, Homo sapiens
PLKKPLGAQ

SEQ ID NO: 199 - protein, 9 aa, Homo sapiens
LKKPLGAQL

SEQ ID NO: 200 - protein, 9 aa, Homo sapiens
KKPLGAQLI

SEQ ID NO: 201 - protein, 9 aa, Homo sapiens
KPLGAQLIT

SEQ ID NO: 202 - protein, 9 aa, Homo sapiens
PLGAQLITM

SEQ ID NO: 203 - protein, 9 aa, Homo sapiens
LGAQLITMD

SEQ ID NO: 204 - protein, 9 aa, Homo sapiens
GAQLITMDW

SEQ ID NO: 205 - protein, 9 aa, Homo sapiens
AQLITMDWT

SEQ ID NO: 206 - protein, 9 aa, Homo sapiens
QLITMDWTW

SEQ ID NO: 207 - protein, 9 aa, Homo sapiens
LITMDWTWR

SEQ ID NO: 208 - protein, 9 aa, Homo sapiens
ITMDWTWRF

SEQ ID NO: 209 - protein, 9 aa, Homo sapiens
TMDWTWRFL

SEQ ID NO: 210 - protein, 9 aa, Homo sapiens
MDWTWRFLF

SEQ ID NO: 211 - protein, 9 aa, Homo sapiens
DWTWRFLFV

SEQ ID NO: 212 - protein, 9 aa, Homo sapiens
WTWRFLFVV

SEQ ID NO: 213 - protein, 9 aa, Homo sapiens
TWRFLFVVA

SEQ ID NO: 214 - protein, 9 aa, Homo sapiens
WRFLFVVAA

SEQ ID NO: 215 - protein, 9 aa, Homo sapiens
RFLFVVAAA

SEQ ID NO: 216 - protein, 9 aa, Homo sapiens
FLFVVAAAT

SEQ ID NO: 217 - protein, 9 aa, Homo sapiens
LFVVAAATG

SEQ ID NO: 218 - protein, 9 aa, Homo sapiens
FVVAAATGV

SEQ ID NO: 219 - protein, 9 aa, Homo sapiens
VVAAATGVQ

SEQ ID NO: 220 - protein, 9 aa, Homo sapiens
VAAATGVQS

SEQ ID NO: 221 - protein, 9 aa, Homo sapiens
AAATGVQSQ

SEQ ID NO: 222 - protein, 9 aa, Homo sapiens
AATGVQSQV

SEQ ID NO: 223 - protein, 9 aa, Homo sapiens
ATGVQSQVQ

SEQ ID NO: 224 - protein, 9 aa, Homo sapiens
TGVQSQVQL

SEQ ID NO: 225 - protein, 9 aa, Homo sapiens
GVQSQVQLV

SEQ ID NO: 226 - protein, 9 aa, Homo sapiens
VQSQVQLVQ

SEQ ID NO: 227 - protein, 9 aa, Homo sapiens
QSQVQLVQS

SEQ ID NO: 228 - protein, 9 aa, Homo sapiens
SQVQLVQSG

SEQ ID NO: 229 - protein, 9 aa, Homo sapiens
QVQLVQSGA

SEQ ID NO: 230 - protein, 9 aa, Homo sapiens
VQLVQSGAE

SEQ ID NO: 231 - protein, 9 aa, Homo sapiens
QLVQSGAEV

SEQ ID NO: 232 - protein, 9 aa, Homo sapiens
LVQSGAEVK

SEQ ID NO: 233 - protein, 9 aa, Homo sapiens
VQSGAEVKK

SEQ ID NO: 234 - protein, 9 aa, Homo sapiens
QSGAEVKKP

SEQ ID NO: 235 - protein, 9 aa, Homo sapiens
SGAEVKKPG

SEQ ID NO: 236 - protein, 9 aa, Homo sapiens
GAEVKKPGS

SEQ ID NO: 237 - protein, 9 aa, Homo sapiens
AEVKKPGSS

SEQ ID NO: 238 - protein, 9 aa, Homo sapiens
EVKKPGSSV

SEQ ID NO: 239 - protein, 9 aa, Homo sapiens
VKKPGSSVK

SEQ ID NO: 240 - protein, 9 aa, Homo sapiens
KKPGSSVKV

SEQ ID NO: 241 - protein, 9 aa, Homo sapiens
KPGSSVKVS

SEQ ID NO: 242 - protein, 9 aa, Homo sapiens
PGSSVKVSC

SEQ ID NO: 243 - protein, 15 aa, Homo sapiens
SGHIPPLKKPLGAQL

SEQ ID NO: 244 - protein, 15 aa, Homo sapiens
GHIPPLKKPLGAQLI

SEQ ID NO: 245 - protein, 15 aa, Homo sapiens
HIPPLKKPLGAQLIT

SEQ ID NO: 246 - protein, 15 aa, Homo sapiens
IPPLKKPLGAQLITM

SEQ ID NO: 247 - protein, 15 aa, Homo sapiens
PPLKKPLGAQLITMD

SEQ ID NO: 248 - protein, 15 aa, Homo sapiens
PLKKPLGAQLITMDW

SEQ ID NO: 249 - protein, 15 aa, Homo sapiens
LKKPLGAQLITMDWT

SEQ ID NO: 250 - protein, 15 aa, Homo sapiens
KKPLGAQLITMDWTW

SEQ ID NO: 251 - protein, 15 aa, Homo sapiens
KPLGAQLITMDWTWR

SEQ ID NO: 252 - protein, 15 aa, Homo sapiens
PLGAQLITMDWTWRF

SEQ ID NO: 253 - protein, 15 aa, Homo sapiens
LGAQLITMDWTWRFL

SEQ ID NO: 254 - protein, 15 aa, Homo sapiens
GAQLITMDWTWRFLF

SEQ ID NO: 255 - protein, 15 aa, Homo sapiens
AQLITMDWTWRFLFV

SEQ ID NO: 256 - protein, 15 aa, Homo sapiens
QLITMDWTWRFLFVV

SEQ ID NO: 257 - protein, 15 aa, Homo sapiens
LITMDWTWRFLFVVA

SEQ ID NO: 258 - protein, 15 aa, Homo sapiens
ITMDWTWRFLFVVAA

SEQ ID NO: 259 - protein, 15 aa, Homo sapiens
TMDWTWRFLFVVAAA

SEQ ID NO: 260 - protein, 15 aa, Homo sapiens
MDWTWRFLFVVAAAT

SEQ ID NO: 261 - protein, 15 aa, Homo sapiens
DWTWRFLFVVAAATG

SEQ ID NO: 262 - protein, 15 aa, Homo sapiens
WTWRFLFVVAAATGV

SEQ ID NO: 263 - protein, 15 aa, Homo sapiens
TWRFLFVVAAATGVQ

SEQ ID NO: 264 - protein, 15 aa, Homo sapiens
WRFLFVVAAATGVQS

SEQ ID NO: 265 - protein, 15 aa, Homo sapiens
RFLFVVAAATGVQSQ

SEQ ID NO: 266 - protein, 15 aa, Homo sapiens
FLFVVAAATGVQSQV

SEQ ID NO: 267 - protein, 15 aa, Homo sapiens
LFVVAAATGVQSQVQ

SEQ ID NO: 268 - protein, 15 aa, Homo sapiens
FVVAAATGVQSQVQL

SEQ ID NO: 269 - protein, 15 aa, Homo sapiens
VVAAATGVQSQVQLV

SEQ ID NO: 270 - protein, 15 aa, Homo sapiens
VAAATGVQSQVQLVQ

SEQ ID NO: 271 - protein, 15 aa, Homo sapiens
AAATGVQSQVQLVQS

SEQ ID NO: 272 - protein, 15 aa, Homo sapiens
AATGVQSQVQLVQSG

SEQ ID NO: 273 - protein, 15 aa, Homo sapiens
ATGVQSQVQLVQSGA

SEQ ID NO: 274 - protein, 15 aa, Homo sapiens
TGVQSQVQLVQSGAE

SEQ ID NO: 275 - protein, 15 aa, Homo sapiens
GVQSQVQLVQSGAEV

SEQ ID NO: 276 - protein, 15 aa, Homo sapiens
VQSQVQLVQSGAEVK

SEQ ID NO: 277 - protein, 15 aa, Homo sapiens
QSQVQLVQSGAEVKK

SEQ ID NO: 278 - protein, 15 aa, Homo sapiens
SQVQLVQSGAEVKKP

SEQ ID NO: 279 - protein, 15 aa, Homo sapiens
QVQLVQSGAEVKKPG

SEQ ID NO: 280 - protein, 15 aa, Homo sapiens
VQLVQSGAEVKKPGS

SEQ ID NO: 281 - protein, 15 aa, Homo sapiens
QLVQSGAEVKKPGSS

SEQ ID NO: 282 - protein, 15 aa, Homo sapiens
LVQSGAEVKKPGSSV

SEQ ID NO: 283 - protein, 15 aa, Homo sapiens
VQSGAEVKKPGSSVK

SEQ ID NO: 284 - protein, 15 aa, Homo sapiens
QSGAEVKKPGSSVKV

SEQ ID NO: 285 - protein, 15 aa, Homo sapiens
SGAEVKKPGSSVKVS

SEQ ID NO: 286 - protein, 15 aa, Homo sapiens
GAEVKKPGSSVKVSC

SEQ ID NO: 287 - protein, 15 aa, Homo sapiens
AEVKKPGSSVKVSCK

SEQ ID NO: 288 - protein, 15 aa, Homo sapiens
EVKKPGSSVKVSCKA

SEQ ID NO: 289 - protein, 15 aa, Homo sapiens
VKKPGSSVKVSCKAT

SEQ ID NO: 290 - protein, 15 aa, Homo sapiens
KKPGSSVKVSCKATG

SEQ ID NO: 291 - protein, 15 aa, Homo sapiens
KPGSSVKVSCKATGG

SEQ ID NO: 292 - protein, 15 aa, Homo sapiens
PGSSVKVSCKATGGT

SEQ ID NO: 293 - protein, 15 aa, Homo sapiens
SGHIPPLKKPLGAQL

SEQ ID NO: 294 - protein, 15 aa, Homo sapiens
GHIPPLKKPLGAQLI

SEQ ID NO: 295 - protein, 15 aa, Homo sapiens
HIPPLKKPLGAQLIT

SEQ ID NO: 296 - protein, 15 aa, Homo sapiens
IPPLKKPLGAQLITM

SEQ ID NO: 297 - protein, 15 aa, Homo sapiens
PPLKKPLGAQLITMD

SEQ ID NO: 298 - protein, 15 aa, Homo sapiens
PLKKPLGAQLITMDW

SEQ ID NO: 299 - protein, 15 aa, Homo sapiens
LKKPLGAQLITMDWT

SEQ ID NO: 300 - protein, 15 aa, Homo sapiens
KKPLGAQLITMDWTW

SEQ ID NO: 301 - protein, 15 aa, Homo sapiens
KPLGAQLITMDWTWR

SEQ ID NO: 302 - protein, 15 aa, Homo sapiens
PLGAQLITMDWTWRF

SEQ ID NO: 303 - protein, 15 aa, Homo sapiens
LGAQLITMDWTWRFL

SEQ ID NO: 304 - protein, 15 aa, Homo sapiens
GAQLITMDWTWRFLF

SEQ ID NO: 305 - protein, 15 aa, Homo sapiens
AQLITMDWTWRFLFV

SEQ ID NO: 306 - protein, 15 aa, Homo sapiens
QLITMDWTWRFLFVV

SEQ ID NO: 307 - protein, 15 aa, Homo sapiens
LITMDWTWRFLFVVA

SEQ ID NO: 308 - protein, 15 aa, Homo sapiens
ITMDWTWRFLFVVAA

SEQ ID NO: 309 - protein, 15 aa, Homo sapiens
TMDWTWRFLFVVAAA

SEQ ID NO: 310 - protein, 15 aa, Homo sapiens
MDWTWRFLFVVAAAT

SEQ ID NO: 311 - protein, 15 aa, Homo sapiens
DWTWRFLFVVAAATG

SEQ ID NO: 312 - protein, 15 aa, Homo sapiens
WTWRFLFVVAAATGV

SEQ ID NO: 313 - protein, 15 aa, Homo sapiens
TWRFLFVVAAATGVQ

SEQ ID NO: 314 - protein, 15 aa, Homo sapiens
WRFLFVVAAATGVQS

SEQ ID NO: 315 - protein, 15 aa, Homo sapiens
RFLFVVAAATGVQSQ

SEQ ID NO: 316 - protein, 15 aa, Homo sapiens
FLFVVAAATGVQSQV

SEQ ID NO: 317 - protein, 15 aa, Homo sapiens
LFVVAAATGVQSQVQ

SEQ ID NO: 318 - protein, 15 aa, Homo sapiens
FVVAAATGVQSQVQL

SEQ ID NO: 319 - protein, 15 aa, Homo sapiens
VVAAATGVQSQVQLV

SEQ ID NO: 320 - protein, 15 aa, Homo sapiens
VAAATGVQSQVQLVQ

SEQ ID NO: 321 - protein, 15 aa, Homo sapiens
AAATGVQSQVQLVQS

SEQ ID NO: 322 - protein, 15 aa, Homo sapiens
AATGVQSQVQLVQSG

SEQ ID NO: 323 - protein, 15 aa, Homo sapiens
ATGVQSQVQLVQSGA

SEQ ID NO: 324 - protein, 15 aa, Homo sapiens
TGVQSQVQLVQSGAE

SEQ ID NO: 325 - protein, 15 aa, Homo sapiens
GVQSQVQLVQSGAEV

SEQ ID NO: 326 - protein, 15 aa, Homo sapiens
VQSQVQLVQSGAEVK

SEQ ID NO: 327 - protein, 15 aa, Homo sapiens
QSQVQLVQSGAEVKK

SEQ ID NO: 328 - protein, 15 aa, Homo sapiens
SQVQLVQSGAEVKKP

SEQ ID NO: 329 - protein, 15 aa, Homo sapiens
QVQLVQSGAEVKKPG

SEQ ID NO: 330 - protein, 15 aa, Homo sapiens
VQLVQSGAEVKKPGS

SEQ ID NO: 331 - protein, 15 aa, Homo sapiens
QLVQSGAEVKKPGSS

SEQ ID NO: 332 - protein, 15 aa, Homo sapiens
LVQSGAEVKKPGSSV

SEQ ID NO: 333 - protein, 15 aa, Homo sapiens
VQSGAEVKKPGSSVK

SEQ ID NO: 334 - protein, 15 aa, Homo sapiens
QSGAEVKKPGSSVKV

SEQ ID NO: 335 - protein, 15 aa, Homo sapiens
SGAEVKKPGSSVKVS

SEQ ID NO: 336 - protein, 15 aa, Homo sapiens
GAEVKKPGSSVKVSC

SEQ ID NO: 337 - protein, 15 aa, Homo sapiens
AEVKKPGSSVKVSCK

SEQ ID NO: 338 - protein, 15 aa, Homo sapiens
EVKKPGSSVKVSCKA

SEQ ID NO: 339 - protein, 15 aa, Homo sapiens
VKKPGSSVKVSCKAT

SEQ ID NO: 340 - protein, 15 aa, Homo sapiens
KKPGSSVKVSCKATG

SEQ ID NO: 341 - protein, 15 aa, Homo sapiens
KPGSSVKVSCKATGG

SEQ ID NO: 342 - protein, 15 aa, Homo sapiens
PGSSVKVSCKATGGT

SEQ ID NO: 343 - protein, 9 aa, Homo sapiens
SGHIPPLKK

SEQ ID NO: 344 - protein, 9 aa, Homo sapiens
GHIPPLKKP

SEQ ID NO: 345 - protein, 9 aa, Homo sapiens
HIPPLKKPL

SEQ ID NO: 346 - protein, 9 aa, Homo sapiens
IPPLKKPLG

SEQ ID NO: 347 - protein, 9 aa, Homo sapiens
PPLKKPLGA

SEQ ID NO: 348 - protein, 9 aa, Homo sapiens
PLKKPLGAQ

SEQ ID NO: 349 - protein, 9 aa, Homo sapiens
LKKPLGAQL

SEQ ID NO: 350 - protein, 9 aa, Homo sapiens
KKPLGAQLI

SEQ ID NO: 351 - protein, 9 aa, Homo sapiens
KPLGAQLIT

SEQ ID NO: 352 - protein, 9 aa, Homo sapiens
PLGAQLITM

SEQ ID NO: 353 - protein, 9 aa, Homo sapiens
LGAQLITMD

SEQ ID NO: 354 - protein, 9 aa, Homo sapiens
GAQLITMDW

SEQ ID NO: 355 - protein, 9 aa, Homo sapiens
AQLITMDWT

SEQ ID NO: 356 - protein, 9 aa, Homo sapiens
QLITMDWTW

SEQ ID NO: 357 - protein, 9 aa, Homo sapiens
LITMDWTWR

SEQ ID NO: 358 - protein, 9 aa, Homo sapiens
ITMDWTWRF

SEQ ID NO: 359 - protein, 9 aa, Homo sapiens
TMDWTWRFL

SEQ ID NO: 360 - protein, 9 aa, Homo sapiens
MDWTWRFLF

SEQ ID NO: 361 - protein, 9 aa, Homo sapiens
DWTWRFLFV

SEQ ID NO: 362 - protein, 9 aa, Homo sapiens
WTWRFLFVV

SEQ ID NO: 363 - protein, 9 aa, Homo sapiens
TWRFLFVVA

SEQ ID NO: 364 - protein, 9 aa, Homo sapiens
WRFLFVVAA

SEQ ID NO: 365 - protein, 9 aa, Homo sapiens
RFLFVVAAA

SEQ ID NO: 366 - protein, 9 aa, Homo sapiens
FLFVVAAAT

SEQ ID NO: 367 - protein, 9 aa, Homo sapiens
LFVVAAATG

SEQ ID NO: 368 - protein, 9 aa, Homo sapiens
FVVAAATGV

SEQ ID NO: 369 - protein, 9 aa, Homo sapiens
VVAAATGVQ

SEQ ID NO: 370 - protein, 9 aa, Homo sapiens
VAAATGVQS

SEQ ID NO: 371 - protein, 9 aa, Homo sapiens
AAATGVQSQ

SEQ ID NO: 372 - protein, 9 aa, Homo sapiens
AATGVQSQV

SEQ ID NO: 373 - protein, 9 aa, Homo sapiens
ATGVQSQVQ

SEQ ID NO: 374 - protein, 9 aa, Homo sapiens
TGVQSQVQL

SEQ ID NO: 375 - protein, 9 aa, Homo sapiens
GVQSQVQLV

SEQ ID NO: 376 - protein, 9 aa, Homo sapiens
VQSQVQLVQ

SEQ ID NO: 377 - protein, 9 aa, Homo sapiens
QSQVQLVQS

SEQ ID NO: 378 - protein, 9 aa, Homo sapiens
SQVQLVQSG

SEQ ID NO: 379 - protein, 9 aa, Homo sapiens
QVQLVQSGA

SEQ ID NO: 380 - protein, 9 aa, Homo sapiens
VQLVQSGAE

SEQ ID NO: 381 - protein, 9 aa, Homo sapiens
QLVQSGAEV

SEQ ID NO: 382 - protein, 9 aa, Homo sapiens
LVQSGAEVK

SEQ ID NO: 383 - protein, 9 aa, Homo sapiens
VQSGAEVKK

SEQ ID NO: 384 - protein, 9 aa, Homo sapiens
QSGAEVKKP

SEQ ID NO: 385 - protein, 9 aa, Homo sapiens
SGAEVKKPG

SEQ ID NO: 386 - protein, 9 aa, Homo sapiens
GAEVKKPGS

SEQ ID NO: 387 - protein, 9 aa, Homo sapiens
AEVKKPGSS

SEQ ID NO: 388 - protein, 9 aa, Homo sapiens
EVKKPGSSV

SEQ ID NO: 389 - protein, 9 aa, Homo sapiens
VKKPGSSVK

SEQ ID NO: 390 - protein, 9 aa, Homo sapiens
KKPGSSVKV

SEQ ID NO: 391 - protein, 9 aa, Homo sapiens
KPGSSVKVS

SEQ ID NO: 392 - protein, 9 aa, Homo sapiens
PGSSVKVSC

SEQ ID NO: 393 - protein, 15 aa, Dengue virus
VTVHTGDQHQVGNES

SEQ ID NO: 394 - protein, 15 aa, Dengue virus
KRLEPSWASVKKDLI

SEQ ID NO: 395 - protein, 15 aa, Dengue virus
EVTAKWLWGFLSRNK

SEQ ID NO: 396 - protein, 15 aa, Dengue virus
VTAHTGDQHQVGNES

SEQ ID NO: 397 - protein, 15 aa, Dengue virus
ITVHTGDQHQVGNDT

SEQ ID NO: 398 - protein, 15 aa, Dengue virus
KRLEPSWANVKKDLI

SEQ ID NO: 399 - protein, 9 aa, Flavivirus
KTLVQSQVN

SEQ ID NO: 400 - protein, 9 aa, Flavivirus
EEPQLVQSY

SEQ ID NO: 401 - protein, 15 aa, Flavivirus
NETTNWLWAFLAREK

SEQ ID NO: 402 - protein, 15 aa, Flavivirus
KKLIPSWASVKEDLV

SEQ ID NO: 403 - protein, 9 aa, Homo sapiens
TNMGAQLIR

SEQ ID NO: 404 - protein, 9 aa, Homo sapiens
KTLVQSQVN

SEQ ID NO: 405 - protein, 9 aa, Homo sapiens
EEPQLVQSY

SEQ ID NO: 406 - protein, 9 aa, Homo sapiens
GGCVTITAE

SEQ ID NO: 407 - protein, 9 aa, Homo sapiens
LICVTVSSG

SEQ ID NO: 408 - protein, 9 aa, Homo sapiens
AAVSVFPLL

SEQ ID NO: 409 - protein, 15 aa, Homo sapiens
EVTAKWLWGFLSRNK

SEQ ID NO: 410 - protein, 15 aa, Homo sapiens
VTVHTGDQHQVGNES

SEQ ID NO: 411 - protein, 15 aa, Homo sapiens
KRLEPSWASVKKDLI

SEQ ID NO: 412 - protein, 15 aa, Homo sapiens
SMAMSCIAVGGITLF

SEQ ID NO: 413 - protein, 15 aa, Homo sapiens
CPGTRVTINADCDKR

SEQ ID NO: 414 - protein, 15 aa, Homo sapiens
LATCGGIMLLSLKGK

SEQ ID NO: 415 - protein, 15 aa, Homo sapiens
ELGLPSEGLGALWKW

SEQ ID NO: 416 - protein, 15 aa, Homo sapiens
TSEYVTTSLASISSQ

SEQ ID NO: 417 - protein, 15 aa, Homo sapiens
YRTAPTGSAASLING

SEQ ID NO: 418 - protein, 15 aa, Homo sapiens
VEVQYAGTDGPCKIP

SEQ ID NO: 419 - protein, 15 aa, Homo sapiens
GHSPDGGSNFPIHDQ

SEQ ID NO: 420 - protein, 15 aa, Homo sapiens
WTSGASTSQGTWNRQ

SEQ ID NO: 421 - protein, 15 aa, Homo sapiens
AATTTAFLVCLVKVV

SEQ ID NO: 422 - protein, 15 aa, Homo sapiens
TTTAFLVCLVKVVRG

SEQ ID NO: 423 - protein, 15 aa, Homo sapiens
VTAHTGDQHQVGNES

SEQ ID NO: 424 - protein, 15 aa, Homo sapiens
ITVHTGDQHQVGNDT

SEQ ID NO: 425 - protein, 15 aa, Homo sapiens
LITMDWTWRFLFVVA

SEQ ID NO: 426 - protein, 15 aa, Homo sapiens
VQLVQSGAEVKKPGS

SEQ ID NO: 427 - protein, 15 aa, Homo sapiens
EVTAKWLWGFLSRNK

SEQ ID NO: 428 - protein, 15 aa, Homo sapiens
KRLEPSWASVKKDLI

SEQ ID NO: 429 - protein, 15 aa, Homo sapiens
KRLEPSWASVKKDLI

SEQ ID NO: 430 - protein, 15 aa, Homo sapiens
HQLWATLLSLTFIKT

SEQ ID NO: 431 - protein, 15 aa, Homo sapiens
GLLGRSQVGVGVFQE

SEQ ID NO: 432 - protein, 15 aa, Homo sapiens
EDTMTYKCPRITETE

SEQ ID NO: 433 - protein, 15 aa, Homo sapiens
VTVHTGDQHQVGNES

SEQ ID NO: 434 - protein, 15 aa, Homo sapiens
QLGQIMLLILCTSQI

SEQ ID NO: 435 - protein, 15 aa, Homo sapiens
QDEKGVTQNGRLITA

SEQ ID NO: 436 - protein, 15 aa, Homo sapiens
EVTAKWLWGFLSRNK

SEQ ID NO: 437 - protein, 15 aa, Homo sapiens
IIFILLMLVTPSMAM

SEQ ID NO: 438 - protein, 15 aa, Homo sapiens
GGVFTSVGKLVHQIF

SEQ ID NO: 439 - protein, 15 aa, Homo sapiens
RGPSLRTTTVTGKII

SEQ ID NO: 440 - protein, 15 aa, Homo sapiens
GIVSILLSSLLKNDV

SEQ ID NO: 441 - protein, 15 aa, Homo sapiens
KRLEPSWASVKKDLI

SEQ ID NO: 442 - protein, 15 aa, Homo sapiens
HQLWATLLSLTFIKT

SEQ ID NO: 443 - protein, 15 aa, Homo sapiens
GLLGRSQVGVGVFQE

SEQ ID NO: 444 - protein, 15 aa, Homo sapiens
EDTMTYKCPRITETE

SEQ ID NO: 445 - protein, 15 aa, Homo sapiens
QDEKGVTQNGRLITA

SEQ ID NO: 446 - protein, 15 aa, Homo sapiens
EVTAKWLWGFLSRNK

SEQ ID NO: 447 - protein, 15 aa, Homo sapiens
GGVFTSVGKLVHQIF

SEQ ID NO: 448 - protein, 15 aa, Homo sapiens
GIVSILLSSLLKNDV

SEQ ID NO: 449 - protein, 9 aa, Homo sapiens
NMYADDTAG

SEQ ID NO: 450 - protein, 9 aa, Homo sapiens
GLNSRSTSL

SEQ ID NO: 451 - protein, 15 aa, Homo sapiens
RSVALAPHVGLGLET

SEQ ID NO: 452 - protein, 15 aa, Homo sapiens
WLGLNSRNTSLSMTC

SEQ ID NO: 453 - protein, 15 aa, Homo sapiens
GIGVLLTWLGLNSRS

SEQ ID NO: 454 - protein, 15 aa, Homo sapiens
PNSLEELGDGLAMGI

SEQ ID NO: 455 - protein, 15 aa, Homo sapiens
WFVPSIKSGNDIANC

SEQ ID NO: 456 - protein, 15 aa, Homo sapiens
VSRGTAKLRWFVERN

SEQ ID NO: 457 - protein, 15 aa, Homo sapiens
ITPMMRHTIENTTAN

SEQ ID NO: 458 - protein, 15 aa, Homo sapiens
ETLMLLALIAVLTGG

SEQ ID NO: 459 - protein, 15 aa, Homo sapiens
KEGDQYIYMGQPLNN

SEQ ID NO: 460 - protein, 15 aa, Homo sapiens
SRNSTHEMYWVSCGT

SEQ ID NO: 461 - protein, 15 aa, Homo sapiens
VRSNAAIGAVFVDEN

SEQ ID NO: 462 - protein, 15 aa, Homo sapiens
EEVQVIAVEPGKNPK

SEQ ID NO: 463 - protein, 15 aa, Homo sapiens
DSKAVHADMGYWIES

SEQ ID NO: 464 - protein, 15 aa, Homo sapiens
TIENTTANISLTAIA

SEQ ID NO: 465 - protein, 15 aa, Homo sapiens
LHPASAWTLYAVATT

SEQ ID NO: 466 - protein, 15 aa, Homo sapiens
LGCGRGGWSYYCAGL

SEQ ID NO: 467 - protein, 15 aa, Homo sapiens
KLGYILRDISKIPGG

SEQ ID NO: 468 - protein, 15 aa, Homo sapiens
EFAAGRRSVSGDLIL

SEQ ID NO: 469 - protein, 15 aa, Homo sapiens
AKKQEVVVLGSQEGA

SEQ ID NO: 470 - protein, 15 aa, Homo sapiens
KPRICTREEFTRKVR

SEQ ID NO: 471 - protein, 15 aa, Homo sapiens
PVTVASAAQRRGRIG

SEQ ID NO: 472 - protein, 9 aa, Homo sapiens
AARGYISTR

SEQ ID NO: 473 - protein, 15 aa, Homo sapiens
RRYLPAIVREAIKRK

SEQ ID NO: 474 - protein, 15 aa, Homo sapiens
RAYRHAMEELPDTIE

SEQ ID NO: 475 - protein, 15 aa, Homo sapiens
KPTYERDVDLGAGTR

SEQ ID NO: 476 - protein, 15 aa, Homo sapiens
PKSHTLWSNGVLESE

SEQ ID NO: 477 - protein, 15 aa, Homo sapiens
VDSFSLGLLCISIMI

SEQ ID NO: 478 - protein, 15 aa, Homo sapiens
DSRCPTQGEATLVEE

SEQ ID NO: 479 - protein, 15 aa, Homo sapiens
VFHTMWHVTRGAVLM

SEQ ID NO: 480 - protein, 15 aa, Homo sapiens
GEGLHKLGYILRDIS

SEQ ID NO: 481 - protein, 15 aa, Homo sapiens
RLCIMVGANASDRMG

SEQ ID NO: 482 - protein, 15 aa, Homo sapiens
EGAWKQIQRVETWAL

SEQ ID NO: 483 - protein, 20 aa, Homo sapiens
QGKRLEPSWASVKKDLISYG

SEQ ID NO: 484 - protein, 15 aa, Homo sapiens
FQSHQLWATLLSLTF

SEQ ID NO: 485 - protein, 18 aa, Homo sapiens
SRSTSLSVSLVLVGVVTL

SEQ ID NO: 486 - protein, 20 aa, Homo sapiens
TAKWLWGFLSRNKKPRICTR

SEQ ID NO: 487 - protein, 9 aa, Homo sapiens
LLMLVTPSM

SEQ ID NO: 488 - protein, 15 aa, Homo sapiens
GMVSILASSLLKNDI

SEQ ID NO: 489 - protein, 19 aa, Homo sapiens
GLNSRSTSLLGLNSRSTSL

SEQ ID NO: 490 - protein, 25 aa, Homo sapiens
SLVASVELPNSLEELGDGLAMGIMI

SEQ ID NO: 491 - protein, 15 aa, Homo sapiens
ISKVRSNAAIGAVFQ

SEQ ID NO: 492 - protein, 15 aa, Homo sapiens
WNTGEEVQVIAVEPG

SEQ ID NO: 493 - protein, 15 aa, Homo sapiens
NRAVHADMGYWIESA

SEQ ID NO: 494 - protein, 15 aa, Homo sapiens
TIENTTANISLTAIA

SEQ ID NO: 495 - protein, 10 aa, Homo sapiens
HPASAWTLYA

SEQ ID NO: 496 - protein, 9 aa, Homo sapiens
YILRDVSKK

SEQ ID NO: 497 - protein, 15 aa, Homo sapiens
HAKKQEVAVLGSQEG

SEQ ID NO: 498 - protein, 15 aa, Homo sapiens
GKKKTPRMCTREEFT

SEQ ID NO: 499 - protein, 15 aa, Homo sapiens
KRYLPAIVREAIKRG

SEQ ID NO: 500 - protein, 10 aa, Homo sapiens
HPASAWTLYA

SEQ ID NO: 501 - protein, 15 aa, Homo sapiens
HTMWHVTRGAVLTYN